European Patent Application EP 4 520 831 A1, published March 12, 2025. Title: NOVEL LENTIVIRAL VECTOR PARTICLES. Applicant: FONDAZIONE TELETHON ETS. The sequence listing filed with the application follows.

SEQUENCE LISTING (16 sequences)

SEQ ID NO: 1 - protein, 512 aa, Autographa californica multiple nucleopolyhedrovirus
MVSAIVLYVLLAAAAHSAFAAEHCNAQMKTGPYKIKNLDITPPKETLQKDVEITIVETDYNENVIIGYKGYYQAYAYNGGSLDPNTRVEETMKTLNVGKEDLLMWSIRQQCEVGEELIDRWGSDSDDCFRDNEGRGQWVKGKELVKRQNNNHFAHHTCNKSWRCGISTSKMYSRLECQDDTDECQVYILDAEGNPINVTVDTVLHRDGVSMILKQKSTFTTRQIKAACLLIKDDKNNPESVTREHCLIDNDIYDLSKNTWNCKFNRCIKRKVEHRVKKRPPTWRHNVRAKYTEGDTATKGDLMHIQEELMYENDLLKMNIELMHAHINKLNNMLHDLIVSVAKVDERLIGNLMNNSVSSTFLSDDTFLLMPCTNPPAHTSNCYNNSIYKEGRWVANTDSSQCIDFSNYKELAIDDDVEFWIPTIGNTTYHDSWKDASGWSFIAQQKSNLITTMENTKFGGVGTSLSDITSMAEGELAAKLTSFMFGHVVNFVIILIVILFLYCMIRNRNRQY

SEQ ID NO: 2 - DNA, 1539 bp, Autographa californica multiple nucleopolyhedrovirus
  source 1..1539: mol_type = other DNA
atggtaagcgctattgttttatatgtgcttttggcggcggcggcgcattctgcctttgcggcggagcactgcaacgcgcaaatgaagacgggtccgtacaagattaaaaacttggacattaccccgcccaaggaaacgctgcaaaaggacgtggaaatcaccatcgtggagacggactacaacgaaaacgtgattatcggctacaaggggtactaccaggcgtatgcgtacaacggcggctcgctggatcccaacacacgcgtcgaagaaaccatgaaaacgctgaatgtgggcaaagaggatttgcttatgtggagcatcaggcagcagtgcgaggtgggcgaagagctgatcgaccgttggggcagtgacagcgacgactgttttcgcgacaacgagggccgcggccagtgggtcaaaggcaaagagttggtgaagcggcagaataacaatcactttgcgcaccacacgtgcaacaaatcgtggcgatgcggcatttccacttcgaaaatgtacagcaggctcgagtgccaggacgacacggacgagtgccaggtatacattttggacgctgagggcaaccccatcaacgtgaccgtggacactgtgcttcatcgagacggcgtgagtatgattctcaaacaaaagtctacgttcaccacgcgccaaataaaagctgcgtgtctgctcattaaagatgacaaaaataaccccgagtcggtgacacgcgaacactgtttgattgacaatgatatatatgatctttctaaaaacacgtggaactgcaagtttaacagatgcattaaacgcaaagtcgagcaccgagtcaagaagcggccgcccacttggcgccacaacgttagagccaagtacacagagggagacactgccaccaaaggcgacctgatgcatattcaagaggagctgatgtacgaaaacgatttgctgaaaatgaacattgagctgatgcatgcgcacatcaacaagctaaacaatatgctgcacgacctgatagtctccgtggccaaggtggacgagcgtttgattggcaatctcatgaacaactctgtttcttcaacatttttgtcggacgacacgtttttgctgatgccgtgcaccaatccgccggcacacaccagtaattgctacaacaacagcatctacaaagaagggcgttgggtggccaacacggactcgtcgcaatgcatagattttagcaactacaaggaactagcaattgacgacgacgtcgagttttggatcccgaccatcggcaacacgacctatcacgacagttggaaagatgccagcggctggtcgtttattgcccaacaaaaaagcaacctcataaccaccatggagaacaccaagtttggcggcgtcggcaccagtctgagcgacatcacttccatggctgaaggcgaattggccgctaaattgacttcgttcatgtttggtcatgtagttaactttgtaattatattaattgtgattttatttttgtactgtatgattagaaaccgtaatagacaatattaa

SEQ ID NO: 3 - protein, 323 aa, Homo sapiens
MWPLVAALLLGSACCGSAQLLFNKTKSVEFTFCNDTVVIPCFVTNMEAQNTTEVYVKWKFKGRDIYTFDGALNKSTVPTDFSSAKIEVSQLLKGDASLKMDKSDAVSHTGNYTCEVTELTREGETIIELKYRVVSWFSPNENILIVIFPIFAILLFWGQFGIKTLKYRSGGMDEKTIALLVAGLVITVIVIVGAILFVPGEYSLKNATGLGLIVTSTGILILLHYYVFSTAIGLTSFVIAILVIQVIAYILAVVGLSLCIAACIPMHGPLLISGLSILALAQLLGLVYMKFVASNQKTIQPPRKAVEEPLNAFKESKGMMNDE

SEQ ID NO: 4 - protein, 114 aa, Homo sapiens
LLFNKTKSVEFTFCNDTVVIPCFVTNMEAQNTTEVYVKWKFKGRDIYTFDGALNKSTVPTDFSSAKIEVSQLLKGDASLKMDKSDAVSHTGNYTCEVTELTREGETIIELKYRV

SEQ ID NO: 5 - DNA, 998 bp, Homo sapiens
  source 1..998: mol_type = other DNA
aattcggatccgccaccatgtggcctctcgtggccgctctgctgctcgggagcgcttgttgcggcagcgcccagctgctgttcaacaaaaccaagtccgtcgagttcaccttctgcaacgacacagtggtgatcccctgcttcgtcaccaacatggaggctcagaataccaccgaggtctacgtcaagtggaaattcaagggcagagacatctacaccttcgacggagccctcaacaagagcacagtgcctaccgacttttccagcgccaagattgaggtgagccaactcctgaagggagacgccagcctgaagatggacaagagcgatgccgtcagccacacaggaaactacacctgcgaggtgacagagctcaccagagagggcgagaccatcatcgagctcaaatacagagtggtgtcctggttctcccccaacgagaacatcctcatcgtgatcttccccatcttcgccatcctgctgttctggggccagttcggcatcaaaaccctgaagtatagatccggcggcatggacgagaaaacaatcgccctgctggtggccggcctcgtgattaccgtgatcgtcatcgtgggcgccatcctcttcgtgcccggagagtacagcctcaagaacgccaccggcctgggcctgattgtgacctccacaggcattctgatcctgctgcactactacgtgttcagcacagccattggcctcacaagcttcgtgatcgccatcctggtcatccaggtgatcgcctacatcctcgccgtggtcggactcagcctctgtattgccgcttgcatccccatgcacggacccctcctgatctccggcctcagcattctggctctcgctcagctgctcggcctggtgtacatgaagttcgtcgccagcaaccagaagaccatccaaccccccagaaaggccgtcgaagagcctctgaacgcctttaaggagagcaagggcatgatgaacgacgagtgagcggccgcg

SEQ ID NO: 6 - DNA, 342 bp, Homo sapiens
  source 1..342: mol_type = other DNA
ctgctgttcaacaaaaccaagtccgtcgagttcaccttctgcaacgacacagtggtgatcccctgcttcgtcaccaacatggaggctcagaataccaccgaggtctacgtcaagtggaaattcaagggcagagacatctacaccttcgacggagccctcaacaagagcacagtgcctaccgacttttccagcgccaagattgaggtgagccaactcctgaagggagacgccagcctgaagatggacaagagcgatgccgtcagccacacaggaaactacacctgcgaggtgacagagctcaccagagagggcgagaccatcatcgagctcaaatacagagtg

SEQ ID NO: 7 - DNA, 4371 bp, Homo sapiens
  source 1..4371: mol_type = other DNA
atgcagattgagctgtccacttgtttcttcctgtgcctcctgcgcttctgtttctccgccactcgccggtactaccttggagccgtggagctttcatgggactacatgcagagcgacctgggcgaactccccgtggatgccagattccccccccgcgtgccaaagtccttcccctttaacacctccgtggtgtacaagaaaaccctctttgtcgagttcactgaccacctgttcaacatcgccaagccgcgcccaccttggatgggcctcctgggaccgaccattcaagctgaagtgtacgacaccgtggtgatcaccctgaagaacatggcgtcccaccccgtgtccctgcatgcggtcggagtgtcctactggaaggcctccgaaggagctgagtacgacgaccagactagccagcgggaaaaggaggacgataaagtgttcccgggcggctcgcatacttacgtgtggcaagtcctgaaggaaaacggacctatggcatccgatcctctgtgcctgacttactcctacctttcccatgtggacctcgtgaaggacctgaacagcgggctgattggtgcacttctcgtgtgccgcgaaggttcgctcgctaaggaaaagacccagaccctccataagttcatccttttgttcgctgtgttcgatgaaggaaagtcatggcattccgaaactaagaactcgctgatgcaggaccgggatgccgcctcagcccgcgcctggcctaaaatgcatacagtcaacggatacgtgaatcggtcactgcccgggctcatcggttgtcacagaaagtccgtgtactggcacgtcatcggcatgggcactacgcctgaagtgcactccatcttcctggaagggcacaccttcctcgtgcgcaaccaccgccaggcctctctggaaatctccccgattacctttctgaccgcccagactctgctcatggacctggggcagttccttctcttctgccacatctccagccatcagcacgacggaatggaggcctacgtgaaggtggactcatgcccggaagaacctcagttgcggatgaagaacaacgaggaggccgaggactatgacgacgatttgactgactccgagatggacgtcgtgcggttcgatgacgacaacagccccagcttcatccagattcgcagcgtggccaagaagcaccccaaaacctgggtgcactacatcgcggccgaggaagaagattgggactacgccccgttggtgctggcacccgatgaccggtcgtacaagtcccagtatctgaacaatggtccgcagcggattggcagaaagtacaagaaagtgcggttcatggcgtacactgacgaaacgtttaagacccgggaggccattcaacatgagagcggcattctgggaccactgctgtacggagaggtcggcgataccctgctcatcatcttcaaaaaccaggcctcccggccttacaacatctaccctcacggaatcaccgacgtgcggccactctactcgcggcgcctgccgaagggcgtcaagcacctgaaagacttccctatcctgccgggcgaaatcttcaagtataagtggaccgtcaccgtggaggacgggcccaccaagagcgatcctaggtgtctgactcggtactactccagcttcgtgaacatggaacgggacctggcatcgggactcattggaccgctgctgatctgctacaaagagtcggtggatcaacgcggcaaccagatcatgtccgacaagcgcaacgtgatcctgttctccgtgtttgatgaaaacagatcctggtacctcactgaaaacatccagaggttcctcccaaaccccgcaggagtgcaactggaggaccctgagtttcaggcctcgaatatcatgcactcgattaacggttacgtgttcgactcgctgcagctgagcgtgtgcctccatgaagtcgcttactggtacattctgtccatcggcgcccagactgacttcctgagcgtgttcttttccggttacacctttaagcacaagatggtgtacgaagataccctgaccctgttccctttctccggcgaaacggtgttcatgtcgatggagaacccgggtctgtggattctgggatgccacaacagcgactttcggaaccgcggaatgactgccctgctgaaggtgtcctcatgcgacaagaacaccggagactactacgaggactcctacgaggatatctcagcctacctcctgtccaagaacaacgcgatcgagccgcgcagcttcagccagaacccgcctgtgctgaagaggcaccagcgagaaattacccggaccaccctccaatcggatcaggaggaaatcgactacgacgacaccatctcggtggaaatgaagaaggaagatttcgatatctacgacgaggacgaaaatcagtcccctcgctcattccaaaagaaaactagacactactttatcgccgcggtggaaagactgtgggactatggaatgtcatccagccctcacgtccttcggaaccgggcccagagcggatcggtgcctcagttcaagaaagtggtgttccaggagttcaccgacggcagcttcacccagccgctgtaccggggagaactgaacgaacacctgggcctgctcggtccctacatccgcgcggaagtggaggataacatcatggtgaccttccgtaaccaagcatccagaccttactccttctattcctccctgatctcatacgaggaggaccagcgccaaggcgccgagccccgcaagaacttcgtcaagcccaacgagactaagacctacttctggaaggtccaacaccatatggccccgaccaaggatgagtttgactgcaaggcctgggcctacttctccgacgtggaccttgagaaggatgtccattccggcctgatcgggccgctgctcgtgtgtcacaccaacaccctgaacccagcgcatggacgccaggtcaccgtccaggagtttgctctgttcttcaccatttttgacgaaactaagtcctggtacttcaccgagaatatggagcgaaactgtagagcgccctgcaatatccagatggaagatccgactttcaaggagaactatagattccacgccatcaacgggtacatcatggatactctgccggggctggtcatggcccaggatcagaggattcggtggtacttgctgtcaatgggatcgaacgaaaacattcactccattcacttctccggtcacgtgttcactgtgcgcaagaaggaggagtacaagatggcgctgtacaatctgtaccccggggtgttcgaaactgtggagatgctgccgtccaaggccggcatctggagagtggagtgcctgatcggagagcacctccacgcggggatgtccaccctcttcctggtgtactcgaataagtgccagaccccgctgggcatggcctcgggccacatcagagacttccagatcacagcaagcggacaatacggccaatgggcgccgaagctggcccgcttgcactactccggatcgatcaacgcatggtccaccaaggaaccgttctcgtggattaaggtggacctcctggcccctatgattatccacggaattaagacccagggcgccaggcagaagttctcctccctgtacatctcgcaattcatcatcatgtacagcctggacgggaagaagtggcagacttacaggggaaactccaccggcaccctgatggtctttttcggcaacgtggattcctccggcattaagcacaacatcttcaacccaccgatcatagccagatatattaggctccaccccactcactactcaatccgctcaactcttcggatggaactcatggggtgcgacctgaactcctgctccatgccgttggggatggaatcaaaggctattagcgacgcccagatcaccgcgagctcctacttcactaacatgttcgccacctggagcccctccaaggccaggctgcacttgcagggacggtcaaatgcctggcggccgcaagtgaacaatccgaaggaatggcttcaagtggatttccaaaagaccatgaaagtgaccggagtcaccacccagggagtgaagtcccttctgacctcgatgtatgtgaaggagttcctgattagcagcagccaggacgggcaccagtggaccctgttcttccaaaacggaaaggtcaaggtgttccaggggaaccaggactcgttcacacccgtggtgaactccctggaccccccactgctgacgcggtacttgaggattcatcctcagtcctgggtccatcagattgcattgcgaatggaagtcctgggctgcgaggcccaggacctgtac

SEQ ID NO: 8 - DNA, 1181 bp, Homo sapiens
  source 1..1181: mol_type = other DNA
ctcgaggagctcaccatggctacattctgatgtaaagagatatatcctatacctgggccaaatgtaaacagcctggaaaagtgttaggttaaaaacaaaacaaaataaataaatgaataaatgccaggtggttatgagtgctattgagaaaaatgaagccaagagggatatcagtgatgcaggtgggggtaaagagcttacaacataaatgtggtgttccatatttaaacctcattcaacagggaagattggagctgaaatgtgaaggagttgtgggagtggaactacgtggaaatctgggggaaaggtgttttgggtaaaagaaatagcaagtgttgaggtccaggggcatgagtgtgcttgatattttagggaagagtaaggagaccagtataaccagagtgagatgagactacagaggtcaggagaaagggcatgcagaccatgtgggatgctctaggacctaggccatggtaaagatgtagggttttaccctgatggaggtcagaagccattggaggattctgagaagaggagtgacaggactcgctttatagttttaaattataactataaattatagtttttaaaacaatagttgcctaacctcatgttatatgtaaaactacagttttaaaaactataaattcctcatactggcagcagtgtgaggggcaagggcaaaagcagagagactaacaggttgctggttactcttgctagtgcaagtgaattctagaatcttcgacaacatccagaacttctcttgctgctgccactcaggaagagggttggagtaggctaggaataggagcacaaattaaagctcctgttcactttgacttctccatccctctcctcctttccttaaaggttctgattaaagcagacttatgcccctactgctctcagaagtgaatgggttaagtttagcagcctcccttttgctacttcagttcttcctgtggctgcttcccactgataaaaaggaagcaatcctatcggttactgcttagtgctgagcacatccagtgggtaaagttccttaaaatgctctgcaaagaaattgggacttttcattaaatcagaaattttacttttttcccctcctgggagctaaagatattttagagaagaattaaccttttgcttctccagttgaacatttgtagcaataagtc

SEQ ID NO: 9 - DNA, 1175 bp, Homo sapiens
  source 1..1175: mol_type = other DNA
gagctcaccatggctacattctgatgtaaagagatatatcctatacctgggccaaatgtaaacagcctggaaaagtgttaggttaaaaacaaaacaaaataaataaatgaataaatgccaggtggttatgagtgctattgagaaaaatgaagccaagagggatatcagtgatgcaggtgggggtaaagagcttacaacataaatgtggtgttccatatttaaacctcattcaacagggaagattggagctgaaatgtgaaggagttgtgggagtggaactacgtggaaatctgggggaaaggtgttttgggtaaaagaaatagcaagtgttgaggtccaggggcatgagtgtgcttgatattttagggaagagtaaggagaccagtataaccagagtgagatgagactacagaggtcaggagaaagggcatgcagaccatgtgggatgctctaggacctaggccatggtaaagatgtagggttttaccctgatggaggtcagaagccattggaggattctgagaagaggagtgacaggactcgctttatagttttaaattataactataaattatagtttttaaaacaatagttgcctaacctcatgttatatgtaaaactacagttttaaaaactataaattcctcatactggcagcagtgtgaggggcaagggcaaaagcagagagactaacaggttgctggttactcttgctagtgcaagtgaattctagaatcttcgacaacatccagaacttctcttgctgctgccactcaggaagagggttggagtaggctaggaataggagcacaaattaaagctcctgttcactttgacttctccatccctctcctcctttccttaaaggttctgattaaagcagacttatgcccctactgctctcagaagtgaatgggttaagtttagcagcctcccttttgctacttcagttcttcctgtggctgcttcccactgataaaaaggaagcaatcctatcggttactgcttagtgctgagcacatccagtgggtaaagttccttaaaatgctctgcaaagaaattgggacttttcattaaatcagaaattttacttttttcccctcctgggagctaaagatattttagagaagaattaaccttttgcttctccagttgaacatttgtagcaataagtc

SEQ ID NO: 10 - DNA, 599 bp, Homo sapiens
  source 1..599: mol_type = other DNA
gtttttaaaacaatagttgcctaacctcatgttatatgtaaaactacagttttaaaaactataaattcctcatactggcagcagtgtgaggggcaagggcaaaagcagagagactaacaggttgctggttactcttgctagtgcaagtgaattctagaatcttcgacaacatccagaacttctcttgctgctgccactcaggaagagggttggagtaggctaggaataggagcacaaattaaagctcctgttcactttgacttctccatccctctcctcctttccttaaaggttctgattaaagcagacttatgcccctactgctctcagaagtgaatgggttaagtttagcagcctcccttttgctacttcagttcttcctgtggctgcttcccactgataaaaaggaagcaatcctatcggttactgcttagtgctgagcacatccagtgggtaaagttccttaaaatgctctgcaaagaaattgggacttttcattaaatcagaaattttacttttttcccctcctgggagctaaagatattttagagaagaattaaccttttgcttctccagttgaacatttgtagcaataagtc

SEQ ID NO: 11 - DNA, 342 bp, Homo sapiens
  source 1..342: mol_type = other DNA
tgacttctccatccctctcctcctttccttaaaggttctgattaaagcagacttatgcccctactgctctcagaagtgaatgggttaagtttagcagcctcccttttgctacttcagttcttcctgtggctgcttcccactgataaaaaggaagcaatcctatcggttactgcttagtgctgagcacatccagtgggtaaagttccttaaaatgctctgcaaagaaattgggacttttcattaaatcagaaattttacttttttcccctcctgggagctaaagatattttagagaagaattaaccttttgcttctccagttgaacatttgtagcaataagtc

SEQ ID NO: 12 - DNA, 4429 bp, Homo sapiens
  source 1..4429: mol_type = other DNA
tcgccaccacttggcttccggcacgtggggcagatgtttccattcccacggcggcagcggaagagggagggccgggcgcgccgcggctgcttgcagtctccgcaagcggctacatcacagagctcagcgtgcggtgtcacaggccccgcggtcccgcccaacagatgcaccgagatgcgcgtgcgcagaaagcgtcccgggggtgaggctccctccctcgctctccctctactcccgccccactctcccccactttcccccctccacccaccgcggccgtcggggctcgctcgctcagtacctggaggcgagttcctgacgcgactgcgactcaatcctcgcctggtgaagaatattttacctatgactcactgaaaataaagacggctgagtgaccgtgtttgttcatgtaaacattgaacaaatatttatcggcttctgcgatgtgtcctactcttttagtggaggaagacacattttatttatgtatttaatttttcttttgaattttacatgcgagttatacttaataaaactcacttcaaaatataccttcaacagaaaatccagcaacagtttctattatgttagttaaaacagccagtcttttcctttacttttaaaaattattcataaatgtaattagtgaatgataataaacattgacatctgatccactgctttaggagtgacacaaatgaagttaactcaggctattttctttataatcattgtgctattgttttctttttcttttcaattatactgcttaatataggattttgtggcaccataggagttgagtaaaaataaaaggaataaaaatataccttatctggccgggcgcggtggctcacgcctgtaatttcagcagtttcggaggccgaggcgggcggatcacgcggtcaggagatcgaggccatcctggctaacatggtgaaaccccgtctctactaaaaatacaaaaaattagccgggcatggtggcggccgcctgtagtcccagctactcgggaggctgaggcaggagaatggcgtgaacccgggaggcggagcttgcagtgagccgagatcgcgacactgcactccagcctgggcgacagagtgagactgcgtctccaaaaaaaaaagaaaaaatacgttatctatgaagatttccaatttgatttctatttatcacaaatggccacagtactcctttgtactttaccacataccatattgtattcagtaattatttgtgaatatgtaattgataatattgtaggttttagagaatccttgaaaacatgaaaatttggtaatggggtctattttgattatttatttatttatttatttattttatttttgagacagagtctcgctcttgttgcccaggctggagtgcagtggcgcgatctcggctcactgcaagctccacctcccgggttcaagcgattctcctgcctcagcctcccaagtagctgggactacaggcacgtgccaccatgcccggctaattttttgtatttttagtagaggaggagtttcatcttgttagctaggatggtctagatctcctgacctcgtgatctgcccgcctcagcctcccaaagtgctgggattacaggtgtgagccaccgtgcccggccatattttgatttaaaatttagcaataatagataaaattttcaatcaactaagcccttgggccagggaatgctattccttaaaaagtgcttctatcaatatagcctctgactcattactttgttaatttttaaattgtatttcattcctgattaacattcccacccagattattaattatacaatctgttaactgtagaacctcaaacatgttggattgtactgtatttgtctggaagacacatttttaaaacattgtaatcgctataagagaagcactgggaaagaaaggagcttctatgcctgcagtgcctgaggagccctttaacagtgtgccccgcccctaagctactcatgcagtcatccccatcccagttagtcaactttattccaaaaaacttggtgttccaaatttttccttctcaaagcccacagatccaaaattcatcagcagttcccacaaacgttaccctcacaatgaatccagccatttttcaccctctccagtggtaccatcatagcccaagccgccaccatttctcacccccggttaacaggccaccctccttctacccttatcctgctagagtttgttttatctacagtgatcagaaagatcagcctaaaagataattctgatcaccaccctcctctactcacaacccggccgtgtctccccattgccctcagtgtagaagtcaatgtccctttgctgaaatgcaaccttagtgaaactttccatgactaacctcctttaaaattgcaacctggtccacccttactcccccttaccccacttctcttttttgcacagcacttattttaccttctaacatactgtataatgtactcatgtattgtaattattgcttatcatccctctttcagttgcttatatttttcatcaatgtgtacccagtgcctaggacaatatctgtctaggacaaatgggtagttatgtggctgtaggcaagccatttaacctctctgtacctcagttactttatctgtatccactttgcggtgttgtcatgaggattaaatcagatagcctatgtgtagcacctggcagtgaatttatcaccctgtactgtaactgtctacttttctgtctcctccattggactgtcattcccagggggttgggaactgggatttcttcatttctgaggcatagaagtatagcatagtggttaggagcatgacttctggagccagagtacatgggtttgaatgctaccactcacaagctgtgtggccatggagaagttgcctaacctctccgtgcttcagtttcatcacccataaaatgaaggtaagaatagtacctgtatttaaaagcacctagaacagttcctggcatatagtgtcagctgtcatctctgcatccttgtacctgtcagagaggagtgtttatcaaaggggcttcttgctgcctgtttccaaaccagtcgacaatataccaattgctccctaacacattcttgtttgtgcagaactgagctcaatgataacatttttatagcaaccctgatcaagtttcttctcataatctcttacactttgaggcccctgcaggggccctcactctccctaataaacattaacctgagtagggtgtttgagctcaccatggctacattctgatgtaaagagatatatcctatacctgggccaaatgtaaacagcctggaaaagtgttaggttaaaaacaaaacaaaataaataaatgaataaatgccaggtggttatgagtgctattgagaaaaatgaagccaagagggatatcagtgatgcaggtgggggtaaagagcttacaacataaatgtggtgttccatatttaaacctcattcaacagggaagattggagctgaaatgtgaaggagttgtgggagtggaactacgtggaaatctgggggaaaggtgttttgggtaaaagaaatagcaagtgttgaggtccaggggcatgagtgtgcttgatattttagggaagagtaaggagaccagtataaccagagtgagatgagactacagaggtcaggagaaagggcatgcagaccatgtgggatgctctaggacctaggccatggtaaagatgtagggttttaccctgatggaggtcagaagccattggaggattctgagaagaggagtgacaggactcgctttatagttttaaattataactataaattatagtttttaaaacaatagttgcctaacctcatgttatatgtaaaactacagttttaaaaactataaattcctcatactggcagcagtgtgaggggcaagggcaaaagcagagagactaacaggttgctggttactcttgctagtgcaagtgaattctagaatcttcgacaacatccagaacttctcttgctgctgccactcaggaagagggttggagtaggctaggaataggagcacaaattaaagctcctgttcactttgacttctccatccctctcctcctttccttaaaggttctgattaaagcagacttatgcccctactgctctcagaagtgaatgggttaagtttagcagcctcccttttgctacttcagttcttcctgtggctgcttcccactgataaaaaggaagcaatcctatcggttactgcttagtgctgagcacatccagtgggtaaagttccttaaaatgctctgcaaagaaattgggacttttcattaaatcagaaattttacttttttcccctcctgggagctaaagatattttagagaagaattaaccttttgcttctccagttgaacatttgtagcaataagtc

SEQ ID NO: 13 - DNA, 523 bp, Homo sapiens
  source 1..523: mol_type = other DNA
ggggctcgctcgctcagtacctggaggcgagttcctgacgcgactgcgactcaatcctcgcctggtgaagaatattttacctatgactcactgaaaataaagacggctgagtgaccgtgtttgttcatgtaaacattgaacaaatatttatcggcttctgcgatgtgtcctactcttttagtggaggaagacacattttatttatgtatttaatttttcttttgaattttacatgcgagttatacttaataaaactcacttcaaaatataccttcaacagaaaatccagcaacagtttctattatgttagttaaaacagccagtcttttcctttacttttaaaaattattcataaatgtaattagtgaatgataataaacattgacatctgatccactgctttaggagtgacacaaatgaagttaactcaggctattttctttataatcattgtgctattgttttctttttcttttcaattatactgcttaatataggattttgtggcaccataggagttgag

SEQ ID NO: 14 - DNA, 804 bp, Homo sapiens
  source 1..804: mol_type = other DNA
tcgccaccacttggcttccggcacgtggggcagatgtttccattcccacggcggcagcggaagagggagggccgggcgcgccgcggctgcttgcagtctccgcaagcggctacatcacagagctcagcgtgcggtgtcacaggccccgcggtcccgcccaacagatgcaccgagatgcgcgtgcgcagaaagcgtcccgggggtgaggctccctccctcgctctccctctactcccgccccactctcccccactttcccccctccacccaccgcggccgtcggggctcgctcgctcagtacctggaggcgagttcctgacgcgactgcgactcaatcctcgcctggtgaagaatattttacctatgactcactgaaaataaagacggctgagtgaccgtgtttgttcatgtaaacattgaacaaatatttatcggcttctgcgatgtgtcctactcttttagtggaggaagacacattttatttatgtatttaatttttcttttgaattttacatgcgagttatacttaataaaactcacttcaaaatataccttcaacagaaaatccagcaacagtttctattatgttagttaaaacagccagtcttttcctttacttttaaaaattattcataaatgtaattagtgaatgataataaacattgacatctgatccactgctttaggagtgacacaaatgaagttaactcaggctattttctttataatcattgtgctattgttttctttttcttttcaattatactgcttaatataggattttgtggcaccataggagttgag

SEQ ID NO: 15 - DNA, 1238 bp, Homo sapiens
  source 1..1238: mol_type = other DNA
cgtttccatcatggtttccaatagaattgagaataccatctattatttatttattcattaaatattgattgtttcagcagcagagggcagtggttgacagtactggctctggagccacatagtttgaatactagatttaccacctattagctgtgtggccttggataaattccttaacctctctgcctcagtttcctcctctgtaaaatgagaagaatcatcctgttttaccaagtactgtgagaattaaacaactaaatccatggagaggcctagaatagtgactagcatgtagtaagttttcaaaaagtgatggctactatccttaactgttttcattattttgaagtgcaggtctctgctctaggaatcaaggggtacagagaagatgaggctatattcttctgtcctcaaggcattcatagctgggcatgggagacagacagatagatgtgacctcggctttcatggctttatgtgcaaaattgtgggagcatcttcagggtcctgtggaggggcagcacaggaaggcttcctggaaggggtggctttagatctggaacttaaagggtaagattgaacctacaggctcagtcacttgttactgaagtggcatggaaaagaagaaagaatgagtcaaaaacccacctgtcagcatctgcaaggagactttttttgcagtagaggttatccagggtgaagccaccacctcctgcaaggtttctgcaacattcattccatacctgggaccgtgctcacttatgggcactcccccaaccccgctcgacagcaagcttggacctttgcattggcaccaaaaggcctgcagtgttccatggcgtggttgtggaaacattgacagggccgcagggcagcagtaggcaggactagaggagggggcagagtagaggagaggcaggaccgttctgagagcttcgcaggcacaaaaatcccgggccaagcctctgcctcagcccctgcaggatatcctgtcattcagcaggatatatagaccatttacagtggccaatttcaccaagactcctggatttgccatttttcctttctgaaggcaggtctcacctatctcctggttcgatctaggaaaaaggaaaggaagggatttaaaagtaaacagtgaaatgagaaagaattcactgggagtttatcaaactaagttaaaatagctaagtcagcctgacaggtgcttggcacagagaaggagcaaatatttcctc

SEQ ID NO: 16 - DNA, 334 bp, Homo sapiens
  source 1..334: mol_type = other DNA
gtagaggagaggcaggaccgttctgagagcttcgcaggcacaaaaatcccgggccaagcctctgcctcagcccctgcaggatatcctgtcattcagcaggatatatagaccatttacagtggccaatttcaccaagactcctggatttgccatttttcctttctgaaggcaggtctcacctatctcctggttcgatctaggaaaaaggaaaggaagggatttaaaagtaaacagtgaaatgagaaagaattcactgggagtttatcaaactaagttaaaatagctaagtcagcctgacaggtgcttggcacagagaaggagcaaatatttcctc